European Patent Application EP 4 649 961 A2, published November 19, 2025. Title: METHODS AND COMPOSITIONS FOR TREATING ANEMIA USING ACTRIIB LIGAND TRAPS AND mTOR INHIBITORS. Applicant: Celgene Corporation. Application EP. The sequence listing filed with the application follows.

SEQUENCE LISTING (34 sequences)

SEQ ID NO: 1 - protein, 106 aa, synthetic construct
  REGION 1..106: note = human ActRIIB soluble (extracellular processed polypeptide with the N-terminal 6 aa of the EC domain deleted and the C-terminal 4 aa of the EC domain deleted (aa 25-130 of SEQ ID NO:14) and with an L79D mutation
ETRECIYYNANWELERTNQSGLERCEGEQDKRLHCYASWRNSSGTIELVKKGCWDDDFNCYDRQECVATEENPQVYFCCCEGNFCNERFTHLPEAGGPEVTYEPPP

SEQ ID NO: 2 - protein, 512 aa, Homo sapiens
  REGION 1..512: note = human ActRIIB precursor protein sequence (A64)
MTAPWVALALLWGSLWPGSGRGEAETRECIYYNANWELERTNQSGLERCEGEQDKRLHCYASWANSSGTIELVKKGCWLDDFNCYDRQECVATEENPQVYFCCCEGNFCNERFTHLPEAGGPEVTYEPPPTAPTLLTVLAYSLLPIGGLSLIVLLAFWMYRHRKPPYGHVDIHEDPGPPPPSPLVGLKPLQLLEIKARGRFGCVWKAQLMNDFVAVKIFPLQDKQSWQSEREIFSTPGMKHENLLQFIAAEKRGSNLEVELWLITAFHDKGSLTDYLKGNIITWNELCHVAETMSRGLSYLHEDVPWCRGEGHKPSIAHRDFKSKNVLLKSDLTAVLADFGLAVRFEPGKPPGDTHGQVGTRRYMAPEVLEGAINFQRDAFLRIDMYAMGLVLWELVSRCKAADGPVDEYMLPFEEEIGQHPSLEELQEVVVHKKMRPTIKDHWLKHPGLAQLCVTIEECWDHDAEARLSAGCVEERVSLIRRSVNGTTSDCLVSLVTSVTNVDLPPKESSI

SEQ ID NO: 3 - protein, 116 aa, Homo sapiens
  REGION 1..116: note = human ActRIIB soluble (extracellular), processed polypeptide sequence (amino acids 19-134 of SEQ ID NO:2)
SGRGEAETRECIYYNANWELERTNQSGLERCEGEQDKRLHCYASWANSSGTIELVKKGCWLDDFNCYDRQECVATEENPQVYFCCCEGNFCNERFTHLPEAGGPEVTYEPPPTAPT

SEQ ID NO: 4 - protein, 101 aa, synthetic construct
  REGION 1..101: note = human ActRIIB soluble (extracellular) processed polypeptide with the C-terminal 15 aa deleted (aa 19-119 of SEQ ID NO.2)
SGRGEAETRECIYYNANWELERTNQSGLERCEGEQDKRLHCYASWANSSGTIELVKKGCWLDDFNCYDRQECVATEENPQVYFCCCEGNFCNERFTHLPEA

SEQ ID NO: 5 - DNA, 1539 bp, Homo sapiens
  misc_feature 1..1539: note = nucleic acid sequence encoding a human ActRIIB (A64) precursor protein
  source 1..1539: mol_type = genomic DNA
atgacggcgccctgggtggccctcgccctcctctggggatcgctgtggcccggctctgggcgtggggaggctgagacacgggagtgcatctactacaacgccaactgggagctggagcgcaccaaccagagcggcctggagcgctgcgaaggcgagcaggacaagcggctgcactgctacgcctcctgggccaacagctctggcaccatcgagctcgtgaagaagggctgctggctagatgacttcaactgctacgataggcaggagtgtgtggccactgaggagaacccccaggtgtacttctgctgctgtgaaggcaacttctgcaacgagcgcttcactcatttgccagaggctgggggcccggaagtcacgtacgagccacccccgacagcccccaccctgctcacggtgctggcctactcactgctgcccatcgggggcctttccctcatcgtcctgctggccttttggatgtaccggcatcgcaagcccccctacggtcatgtggacatccatgaggaccctgggcctccaccaccatcccctctggtgggcctgaagccactgcagctgctggagatcaaggctcgggggcgctttggctgtgtctggaaggcccagctcatgaatgactttgtagctgtcaagatcttcccactccaggacaagcagtcgtggcagagtgaacgggagatcttcagcacacctggcatgaagcacgagaacctgctacagttcattgctgccgagaagcgaggctccaacctcgaagtagagctgtggctcatcacggccttccatgacaagggctccctcacggattacctcaaggggaacatcatcacatggaacgaactgtgtcatgtagcagagacgatgtcacgaggcctctcatacctgcatgaggatgtgccctggtgccgtggcgagggccacaagccgtctattgcccacagggactttaaaagtaagaatgtattgctgaagagcgacctcacagccgtgctggctgactttggcttggctgttcgatttgagccagggaaacctccaggggacacccacggacaggtaggcacgagacggtacatggctcctgaggtgctcgagggagccatcaacttccagagagatgccttcctgcgcattgacatgtatgccatggggttggtgctgtgggagcttgtgtctcgctgcaaggctgcagacggacccgtggatgagtacatgctgccctttgaggaagagattggccagcacccttcgttggaggagctgcaggaggtggtggtgcacaagaagatgaggcccaccattaaagatcactggttgaaacacccgggcctggcccagctttgtgtgaccatcgaggagtgctgggaccatgatgcagaggctcgcttgtccgcgggctgtgtggaggagcgggtgtccctgattcggaggtcggtcaacggcactacctcggactgtctcgtttccctggtgacctctgtcaccaatgtggacctgccccctaaagagtcaagcatctaa

SEQ ID NO: 6 - protein, 344 aa, synthetic construct
  REGION 1..344: note = fusion protein comprising a soluble extracellular domain of ActRIIB (A64; SEQ ID NO: 3) fused to an Fc domain
SGRGEAETRECIYYNANWELERTNQSGLERCEGEQDKRLHCYASWANSSGTIELVKKGCWLDDFNCYDRQECVATEENPQVYFCCCEGNFCNERFTHLPEAGGPEVTYEPPPTAPTGGGTHTCPPCPAPELLGGPSVFLFPPKPKDTLMISRTPEVTCVVVDVSHEDPEVKFNWYVDGVEVHNAKTKPREEQYNSTYRVVSVLTVLHQDWLNGKEYKCKVSNKALPVPIEKTISKAKGQPREPQVYTLPPSREEMTKNQVSLTCLVKGFYPSDIAVEWESNGQPENNYKTTPPVLDSDGSFFLYSKLTVDKSRWQQGNVFSCSVMHEALHNHYTQKSLSLSPGK

SEQ ID NO: 7 - protein, 329 aa, synthetic construct
  REGION 1..329: note = fusion protein comprising a soluble extracellular domain of ActRIIB (A64) with the C-terminal 15 amino acids deleted (SEQ ID NO:4) fused to an Fc domain
SGRGEAETRECIYYNANWELERTNQSGLERCEGEQDKRLHCYASWANSSGTIELVKKGCWLDDFNCYDRQECVATEENPQVYFCCCEGNFCNERFTHLPEAGGGTHTCPPCPAPELLGGPSVFLFPPKPKDTLMISRTPEVTCVVVDVSHEDPEVKFNWYVDGVEVHNAKTKPREEQYNSTYRVVSVLTVLHQDWLNGKEYKCKVSNKALPVPIEKTISKAKGQPREPQVYTLPPSREEMTKNQVSLTCLVKGFYPSDIAVEWESNGQPENNYKTTPPVLDSDGSFFLYSKLTVDKSRWQQGNVFSCSVMHEALHNHYTQKSLSLSPGK

SEQ ID NO: 8 - protein, 105 aa, synthetic construct
  REGION 1..105: note = human ActRIIB soluble (extracellular) processed polypeptide with the N-terminal 6 aa of the EC domain deleted and the C-terminal 5 aa of the EC domain deleted (aa 25-129 of SEQ ID NO:14) and with an L79D mutation
ETRECIYYNANWELERTNQSGLERCEGEQDKRLHCYASWRNSSGTIELVKKGCWDDDFNCYDRQECVATEENPQVYFCCCEGNFCNERFTHLPEAGGPEVTYEPP

SEQ ID NO: 9 - protein, 107 aa, synthetic construct
  REGION 1..107: note = human ActRIIB soluble (extracellular) processed polypeptide with the N-terminal 6 aa of the EC domain deleted and the C-terminal 3 aa of the EC domain deleted (aa 25-131 of SEQ ID NO:14) and with an L79D mutation
ETRECIYYNANWELERTNQSGLERCEGEQDKRLHCYASWRNSSGTIELVKKGCWDDDFNCYDRQECVATEENPQVYFCCCEGNFCNERFTHLPEAGGPEVTYEPPPT

SEQ ID NO: 10 - protein, 360 aa, synthetic construct
  REGION 1..360: note = Unprocessed ActRIIB-Fc fusion protein with the N-terminal 6 aa of the EC domain deleted and the C-terminal 3 aa of the EC domain deleted (aa 25-131 of SEQ ID NO:14) and with an L79D mutation and with TPA leader sequence
MDAMKRGLCCVLLLCGAVFVSPGAAETRECIYYNANWELERTNQSGLERCEGEQDKRLHCYASWRNSSGTIELVKKGCWDDDFNCYDRQECVATEENPQVYFCCCEGNFCNERFTHLPEAGGPEVTYEPPPTGGGTHTCPPCPAPELLGGPSVFLFPPKPKDTLMISRTPEVTCVVVDVSHEDPEVKFNWYVDGVEVHNAKTKPREEQYNSTYRVVSVLTVLHQDWLNGKEYKCKVSNKALPAPIEKTISKAKGQPREPQVYTLPPSREEMTKNQVSLTCLVKGFYPSDIAVEWESNGQPENNYKTTPPVLDSDGSFFLYSKLTVDKSRWQQGNVFSCSVMHEALHNHYTQKSLSLSPGK

SEQ ID NO: 11 - protein, 335 aa, synthetic construct
  REGION 1..335: note = Processed ActRIIB-Fc fusion protein with the N-terminal 6 aa of the EC domain deleted and the C-terminal 3 aa of the EC domain deleted (aa 25-131 of SEQ ID NO:14) and with an L79D mutation (Luspatercept)
ETRECIYYNANWELERTNQSGLERCEGEQDKRLHCYASWRNSSGTIELVKKGCWDDDFNCYDRQECVATEENPQVYFCCCEGNFCNERFTHLPEAGGPEVTYEPPPTGGGTHTCPPCPAPELLGGPSVFLFPPKPKDTLMISRTPEVTCVVVDVSHEDPEVKFNWYVDGVEVHNAKTKPREEQYNSTYRVVSVLTVLHQDWLNGKEYKCKVSNKALPAPIEKTISKAKGQPREPQVYTLPPSREEMTKNQVSLTCLVKGFYPSDIAVEWESNGQPENNYKTTPPVLDSDGSFFLYSKLTVDKSRWQQGNVFSCSVMHEALHNHYTQKSLSLSPGK

SEQ ID NO: 12 - protein, 115 aa, Homo sapiens
  REGION 1..115: note = human ActRIIB soluble (extracellular), processed polypeptide sequence (amino acids 20-134 of SEQ ID NO:2)
GRGEAETRECIYYNANWELERTNQSGLERCEGEQDKRLHCYASWANSSGTIELVKKGCWLDDFNCYDRQECVATEENPQVYFCCCEGNFCNERFTHLPEAGGPEVTYEPPPTAPT

SEQ ID NO: 13 - protein, 100 aa, synthetic construct
  REGION 1..100: note = human ActRIIB soluble (extracellular), processed polypeptide sequence with the C-terminal 15 aa deleted (aa 20-119 of SEQ ID NO:2)
GRGEAETRECIYYNANWELERTNQSGLERCEGEQDKRLHCYASWANSSGTIELVKKGCWLDDFNCYDRQECVATEENPQVYFCCCEGNFCNERFTHLPEA

SEQ ID NO: 14 - protein, 512 aa, Homo sapiens
  REGION 1..512: note = human ActRIIB precursor protein sequence (R64)
MTAPWVALALLWGSLWPGSGRGEAETRECIYYNANWELERTNQSGLERCEGEQDKRLHCYASWRNSSGTIELVKKGCWLDDFNCYDRQECVATEENPQVYFCCCEGNFCNERFTHLPEAGGPEVTYEPPPTAPTLLTVLAYSLLPIGGLSLIVLLAFWMYRHRKPPYGHVDIHEDPGPPPPSPLVGLKPLQLLEIKARGRFGCVWKAQLMNDFVAVKIFPLQDKQSWQSEREIFSTPGMKHENLLQFIAAEKRGSNLEVELWLITAFHDKGSLTDYLKGNIITWNELCHVAETMSRGLSYLHEDVPWCRGEGHKPSIAHRDFKSKNVLLKSDLTAVLADFGLAVRFEPGKPPGDTHGQVGTRRYMAPEVLEGAINFQRDAFLRIDMYAMGLVLWELVSRCKAADGPVDEYMLPFEEEIGQHPSLEELQEVVVHKKMRPTIKDHWLKHPGLAQLCVTIEECWDHDAEARLSAGCVEERVSLIRRSVNGTTSDCLVSLVTSVTNVDLPPKESSI

SEQ ID NO: 15 - protein, 116 aa, synthetic construct
  REGION 1..116: note = human ActRIIB soluble (extracellular), processed polypeptide sequence (amino acids 19-134 of SEQ ID NO:14)
SGRGEAETRECIYYNANWELERTNQSGLERCEGEQDKRLHCYASWRNSSGTIELVKKGCWLDDFNCYDRQECVATEENPQVYFCCCEGNFCNERFTHLPEAGGPEVTYEPPPTAPT

SEQ ID NO: 16 - protein, 101 aa, synthetic construct
  REGION 1..101: note = human ActRIIB soluble (extracellular), processed polypeptide sequence with the C-terminal 15 aa deleted (aa 19-119 of SEQ ID NO:14)
SGRGEAETRECIYYNANWELERTNQSGLERCEGEQDKRLHCYASWRNSSGTIELVKKGCWLDDFNCYDRQECVATEENPQVYFCCCEGNFCNERFTHLPEA

SEQ ID NO: 17 - protein, 115 aa, synthetic construct
  REGION 1..115: note = human ActRIIB soluble (extracellular), processed polypeptide sequence (amino acids 20-134 of SEQ ID NO:14)
GRGEAETRECIYYNANWELERTNQSGLERCEGEQDKRLHCYASWRNSSGTIELVKKGCWLDDFNCYDRQECVATEENPQVYFCCCEGNFCNERFTHLPEAGGPEVTYEPPPTAPT

SEQ ID NO: 18 - protein, 100 aa, synthetic construct
  REGION 1..100: note = human ActRIIB soluble (extracellular), processed polypeptide sequence with the C-terminal 15 aa deleted (aa 20-119 of SEQ ID NO:14)
GRGEAETRECIYYNANWELERTNQSGLERCEGEQDKRLHCYASWRNSSGTIELVKKGCWLDDFNCYDRQECVATEENPQVYFCCCEGNFCNERFTHLPEA

SEQ ID NO: 19 - protein, 107 aa, synthetic construct
  REGION 1..107: note = human ActRIIB soluble (extracellular) processed polypeptide with the N-terminal 6 aa of the EC domain deleted and the C-terminal 3 aa of the EC domain deleted (aa 25-131 of SEQ ID NO:2) and with an L79D mutation
ETRECIYYNANWELERTNQSGLERCEGEQDKRLHCYASWANSSGTIELVKKGCWDDDFNCYDRQECVATEENPQVYFCCCEGNFCNERFTHLPEAGGPEVTYEPPPT

SEQ ID NO: 20 - protein, 360 aa, synthetic construct
  REGION 1..360: note = Unprocessed ActRIIB-Fc fusion protein with the N-terminal 6 aa of the EC domain deleted and the C-terminal 3 aa of the EC domain deleted (aa 25-131 of SEQ ID NO:2) and with an L79D mutation and with TPA leader sequence
MDAMKRGLCCVLLLCGAVFVSPGAAETRECIYYNANWELERTNQSGLERCEGEQDKRLHCYASWANSSGTIELVKKGCWDDDFNCYDRQECVATEENPQVYFCCCEGNFCNERFTHLPEAGGPEVTYEPPPTGGGTHTCPPCPAPELLGGPSVFLFPPKPKDTLMISRTPEVTCVVVDVSHEDPEVKFNWYVDGVEVHNAKTKPREEQYNSTYRVVSVLTVLHQDWLNGKEYKCKVSNKALPAPIEKTISKAKGQPREPQVYTLPPSREEMTKNQVSLTCLVKGFYPSDIAVEWESNGQPENNYKTTPPVLDSDGSFFLYSKLTVDKSRWQQGNVFSCSVMHEALHNHYTQKSLSLSPGK

SEQ ID NO: 21 - protein, 335 aa, synthetic construct
  REGION 1..335: note = Processed ActRIIB-Fc fusion protein with the N-terminal 6 aa of the EC domain deleted and the C-terminal 3 aa of the EC domain deleted (aa 25-131 of SEQ ID NO:2) and with an L79D mutation
ETRECIYYNANWELERTNQSGLERCEGEQDKRLHCYASWANSSGTIELVKKGCWDDDFNCYDRQECVATEENPQVYFCCCEGNFCNERFTHLPEAGGPEVTYEPPPTGGGTHTCPPCPAPELLGGPSVFLFPPKPKDTLMISRTPEVTCVVVDVSHEDPEVKFNWYVDGVEVHNAKTKPREEQYNSTYRVVSVLTVLHQDWLNGKEYKCKVSNKALPAPIEKTISKAKGQPREPQVYTLPPSREEMTKNQVSLTCLVKGFYPSDIAVEWESNGQPENNYKTTPPVLDSDGSFFLYSKLTVDKSRWQQGNVFSCSVMHEALHNHYTQKSLSLSPGK

SEQ ID NO: 22 - protein, 115 aa, synthetic construct
  REGION 1..115: note = human ActRIIB soluble (extracellular), processed polypeptide sequence (amino acids 20-134 of SEQ ID NO:14) with L79D mutation
GRGEAETRECIYYNANWELERTNQSGLERCEGEQDKRLHCYASWRNSSGTIELVKKGCWDDDFNCYDRQECVATEENPQVYFCCCEGNFCNERFTHLPEAGGPEVTYEPPPTAPT

SEQ ID NO: 23 - protein, 115 aa, synthetic construct
  REGION 1..115: note = human ActRIIB soluble (extracellular), processed polypeptide sequence (amino acids 20-134 of SEQ ID NO:2) with L79D mutation
GRGEAETRECIYYNANWELERTNQSGLERCEGEQDKRLHCYASWANSSGTIELVKKGCWDDDFNCYDRQECVATEENPQVYFCCCEGNFCNERFTHLPEAGGPEVTYEPPPTAPT

SEQ ID NO: 24 - protein, 343 aa, synthetic construct
  REGION 1..343: note = human ActRIIB soluble (extracellular), processed polypeptide sequence (aa 20-134 of SEQ ID NO:14) with L79D mutation fused to an Fc domain with a GGG linker
GRGEAETRECIYYNANWELERTNQSGLERCEGEQDKRLHCYASWRNSSGTIELVKKGCWDDDFNCYDRQECVATEENPQVYFCCCEGNFCNERFTHLPEAGGPEVTYEPPPTAPTGGGTHTCPPCPAPELLGGPSVFLFPPKPKDTLMISRTPEVTCVVVDVSHEDPEVKFNWYVDGVEVHNAKTKPREEQYNSTYRVVSVLTVLHQDWLNGKEYKCKVSNKALPAPIEKTISKAKGQPREPQVYTLPPSREEMTKNQVSLTCLVKGFYPSDIAVEWESNGQPENNYKTTPPVLDSDGSFFLYSKLTVDKSRWQQGNVFSCSVMHEALHNHYTQKSLSLSPGK

SEQ ID NO: 25 - protein, 343 aa, synthetic construct
  REGION 1..343: note = human ActRIIB soluble (extracellular), processed polypeptide sequence (aa 20-134 of SEQ ID NO:2) with L79D mutation fused to an Fc domain
GRGEAETRECIYYNANWELERTNQSGLERCEGEQDKRLHCYASWANSSGTIELVKKGCWDDDFNCYDRQECVATEENPQVYFCCCEGNFCNERFTHLPEAGGPEVTYEPPPTAPTGGGTHTCPPCPAPELLGGPSVFLFPPKPKDTLMISRTPEVTCVVVDVSHEDPEVKFNWYVDGVEVHNAKTKPREEQYNSTYRVVSVLTVLHQDWLNGKEYKCKVSNKALPAPIEKTISKAKGQPREPQVYTLPPSREEMTKNQVSLTCLVKGFYPSDIAVEWESNGQPENNYKTTPPVLDSDGSFFLYSKLTVDKSRWQQGNVFSCSVMHEALHNHYTQKSLSLSPGK

SEQ ID NO: 26 - protein, 368 aa, synthetic construct
  REGION 1..368: note = human ActRIIB soluble (extracellular), processed polypeptide sequence (aa 20-134 of SEQ ID NO:14) with L79D mutation fused to an Fc domain and with TPA leader sequence
MDAMKRGLCCVLLLCGAVFVSPGASGRGEAETRECIYYNANWELERTNQSGLERCEGEQDKRLHCYASWRNSSGTIELVKKGCWDDDFNCYDRQECVATEENPQVYFCCCEGNFCNERFTHLPEAGGPEVTYEPPPTAPTGGGTHTCPPCPAPELLGGPSVFLFPPKPKDTLMISRTPEVTCVVVDVSHEDPEVKFNWYVDGVEVHNAKTKPREEQYNSTYRVVSVLTVLHQDWLNGKEYKCKVSNKALPAPIEKTISKAKGQPREPQVYTLPPSREEMTKNQVSLTCLVKGFYPSDIAVEWESNGQPENNYKTTPPVLDSDGSFFLYSKLTVDKSRWQQGNVFSCSVMHEALHNHYTQKSLSLSPGK

SEQ ID NO: 27 - protein, 368 aa, synthetic construct
  REGION 1..368: note = human ActRIIB soluble (extracellular), processed polypeptide sequence (aa 20-134 of SEQ ID NO:2) with L79D mutation fused to an Fc domain and with TPA leader sequence
MDAMKRGLCCVLLLCGAVFVSPGASGRGEAETRECIYYNANWELERTNQSGLERCEGEQDKRLHCYASWANSSGTIELVKKGCWDDDFNCYDRQECVATEENPQVYFCCCEGNFCNERFTHLPEAGGPEVTYEPPPTAPTGGGTHTCPPCPAPELLGGPSVFLFPPKPKDTLMISRTPEVTCVVVDVSHEDPEVKFNWYVDGVEVHNAKTKPREEQYNSTYRVVSVLTVLHQDWLNGKEYKCKVSNKALPAPIEKTISKAKGQPREPQVYTLPPSREEMTKNQVSLTCLVKGFYPSDIAVEWESNGQPENNYKTTPPVLDSDGSFFLYSKLTVDKSRWQQGNVFSCSVMHEALHNHYTQKSLSLSPGK

SEQ ID NO: 28 - protein, 141 aa, synthetic construct
  REGION 1..141: note = human ActRIIB soluble (extracellular), processed polypeptide sequence having a variant C-terminal sequence (disclosed in WO2007/053775)
GRGEAETRECIYYNANWELERTNQSGLERCEGEQDKRLHCYASWRNSSGTIELVKKGCWLDDFNCYDRQECVATEENPQVYFCCCEGNFCNERFTHLPEAGGPEGPWASTTIPSGGPEATAAAGDQGSGALWLCLEGPAHE

SEQ ID NO: 29 - protein, 141 aa, synthetic construct
  REGION 1..141: note = human ActRIIB soluble (extracellular), processed polypeptide sequence having a variant C-terminal sequence (disclosed in WO2007/053775) having an L79D mutation
GRGEAETRECIYYNANWELERTNQSGLERCEGEQDKRLHCYASWRNSSGTIELVKKGCWDDDFNCYDRQECVATEENPQVYFCCCEGNFCNERFTHLPEAGGPEGPWASTTIPSGGPEATAAAGDQGSGALWLCLEGPAHE

SEQ ID NO: 30 - protein, 370 aa, synthetic construct
  REGION 1..370: note = human ActRIIB soluble (extracellular), processed polypeptide sequence having a variant C-terminal sequence (disclosed in WO2007/053775) having an L79D mutation fused to an Fc domain with a TGGG linker
GRGEAETRECIYYNANWELERTNQSGLERCEGEQDKRLHCYASWRNSSGTIELVKKGCWDDDFNCYDRQECVATEENPQVYFCCCEGNFCNERFTHLPEAGGPEGPWASTTIPSGGPEATAAAGDQGSGALWLCLEGPAHETGGGTHTCPPCPAPELLGGPSVFLFPPKPKDTLMISRTPEVTCVVVDVSHEDPEVKFNWYVDGVEVHNAKTKPREEQYNSTYRVVSVLTVLHQDWLNGKEYKCKVSNKALPAPIEKTISKAKGQPREPQVYTLPPSREEMTKNQVSLTCLVKGFYPSDIAVEWESNGQPENNYKTTPPVLDSDGSFFLYSKLTVDKSRWQQGNVFSCSVMHEALHNHYTQKSLSLSPGK

SEQ ID NO: 31 - DNA, 1083 bp, synthetic construct
  misc_feature 1..1083: note = Nucleic Acid Sequence Encoding SEQ ID NO:10
  source 1..1083: mol_type = other DNA
atggatgcaatgaagagagggctctgctgtgtgctgctgctgtgtggagcagtcttcgtttcgcccggcgccgccgaaacccgcgaatgtatttattacaatgctaattgggaactcgaacggacgaaccaatccgggctcgaacggtgtgagggggaacaggataaacgcctccattgctatgcgtcgtggaggaactcctccgggacgattgaactggtcaagaaagggtgctgggacgacgatttcaattgttatgaccgccaggaatgtgtcgcgaccgaagagaatccgcaggtctatttctgttgttgcgaggggaatttctgtaatgaacggtttacccacctccccgaagccggcgggcccgaggtgacctatgaacccccgcccaccggtggtggaactcacacatgcccaccgtgcccagcacctgaactcctggggggaccgtcagtcttcctcttccccccaaaacccaaggacaccctcatgatctcccggacccctgaggtcacatgcgtggtggtggacgtgagccacgaagaccctgaggtcaagttcaactggtacgtggacggcgtggaggtgcataatgccaagacaaagccgcgggaggagcagtacaacagcacgtaccgtgtggtcagcgtcctcaccgtcctgcaccaggactggctgaatggcaaggagtacaagtgcaaggtctccaacaaagccctcccagcccccatcgagaaaaccatctccaaagccaaagggcagccccgagaaccacaggtgtacaccctgcccccatcccgggaggagatgaccaagaaccaggtcagcctgacctgcctggtcaaaggcttctatcccagcgacatcgccgtggagtgggagagcaatgggcagccggagaacaactacaagaccacgcctcccgtgctggactccgacggctccttcttcctctatagcaagctcaccgtggacaagagcaggtggcagcaggggaacgtcttctcatgctccgtgatgcatgaggctctgcacaaccactacacgcagaagagcctctccctgtccccgggtaaatga

SEQ ID NO: 32 - protein, 344 aa, synthetic construct
  REGION 1..344: note = fusion protein comprising a soluble extracellular domain of ActRIIB (R64; SEQ ID NO:15) fused to an Fc domain
SGRGEAETRECIYYNANWELERTNQSGLERCEGEQDKRLHCYASWRNSSGTIELVKKGCWLDDFNCYDRQECVATEENPQVYFCCCEGNFCNERFTHLPEAGGPEVTYEPPPTAPTGGGTHTCPPCPAPELLGGPSVFLFPPKPKDTLMISRTPEVTCVVVDVSHEDPEVKFNWYVDGVEVHNAKTKPREEQYNSTYRVVSVLTVLHQDWLNGKEYKCKVSNKALPVPIEKTISKAKGQPREPQVYTLPPSREEMTKNQVSLTCLVKGFYPSDIAVEWESNGQPENNYKTTPPVLDSDGSFFLYSKLTVDKSRWQQGNVFSCSVMHEALHNHYTQKSLSLSPGK

SEQ ID NO: 33 - protein, 329 aa, synthetic construct
  REGION 1..329: note = fusion protein comprising a soluble extracellular domain of ActRIIB (R64) with the C-terminal 15 aa deleted (SEQ ID NO:16) fused to an Fc domain
SGRGEAETRECIYYNANWELERTNQSGLERCEGEQDKRLHCYASWRNSSGTIELVKKGCWLDDFNCYDRQECVATEENPQVYFCCCEGNFCNERFTHLPEAGGGTHTCPPCPAPELLGGPSVFLFPPKPKDTLMISRTPEVTCVVVDVSHEDPEVKFNWYVDGVEVHNAKTKPREEQYNSTYRVVSVLTVLHQDWLNGKEYKCKVSNKALPVPIEKTISKAKGQPREPQVYTLPPSREEMTKNQVSLTCLVKGFYPSDIAVEWESNGQPENNYKTTPPVLDSDGSFFLYSKLTVDKSRWQQGNVFSCSVMHEALHNHYTQKSLSLSPGK

SEQ ID NO: 34 - DNA, 1083 bp, synthetic construct
  regulatory 1..72: note = misc_signal - nt sequence encoding TPA signal peptide; regulatory_class = other
  misc_feature 1..1083: note = Nucleic acid sequence that encodes SEQ ID NO:1 and tissue plasminogen activator (TPA signal peptide sequence)
  source 1..1083: mol_type = other DNA
atggatgcaatgaagagagggctctgctgtgtgctgctgctgtgtggagcagtcttcgtttcgcccggcgccgccgaaacccgcgaatgtatttattacaatgctaattgggaactcgaacggacgaaccaatccgggctcgaacggtgtgagggggaacaggataaacgcctccattgctatgcgtcgtggaggaactcctccgggacgattgaactggtcaagaaagggtgctgggacgacgatttcaattgttatgaccgccaggaatgtgtcgcgaccgaagagaatccgcaggtctatttctgttgttgcgaggggaatttctgtaatgaacggtttacccacctccccgaagccggcgggcccgaggtgacctatgaacccccgcccaccggtggtggaactcacacatgcccaccgtgcccagcacctgaactcctggggggaccgtcagtcttcctcttccccccaaaacccaaggacaccctcatgatctcccggacccctgaggtcacatgcgtggtggtggacgtgagccacgaagaccctgaggtcaagttcaactggtacgtggacggcgtggaggtgcataatgccaagacaaagccgcgggaggagcagtacaacagcacgtaccgtgtggtcagcgtcctcaccgtcctgcaccaggactggctgaatggcaaggagtacaagtgcaaggtctccaacaaagccctcccagcccccatcgagaaaaccatctccaaagccaaagggcagccccgagaaccacaggtgtacaccctgcccccatcccgggaggagatgaccaagaaccaggtcagcctgacctgcctggtcaaaggcttctatcccagcgacatcgccgtggagtgggagagcaatgggcagccggagaacaactacaagaccacgcctcccgtgctggactccgacggctccttcttcctctatagcaagctcaccgtggacaagagcaggtggcagcaggggaacgtcttctcatgctccgtgatgcatgaggctctgcacaaccactacacgcagaagagcctctccctgtctccgggtaaatga